European Patent Specification EP 3 538 554 B1, published August 13, 2025. Title: Antigen-Binding Proteins That Antagonize Leptin Receptor. Applicant: Regeneron Pharmaceuticals, Inc. Gromada, Jesper Stevis, Panayiotis Altarejos, Judith. Application TBD. The sequence listing filed with the application follows.

SEQUENCE LISTING (95 sequences)

SEQ ID NO: 1 - DNA, 378 bp, Artificial Sequence
  synthetic
cagctgcagctgcaggagtcgggcccaggactggtgaagccttcggagaccctgtccctcacctgcactgtctctggtgcctctatcagcagtagtcgtttctacgggggctggatccgccagcccccagggaagggtctggagtggattggggatatctattatagtgggaatacctactacaacccgtccctccagagtcgagtcaccatatccgtagacacgtccaagaatcagttctccctgaagctgagctctgtgaccgccgcagacacggctgtgtattactgtgcgagacaccttatgattacgtttgggggacttatcgtcgagggttttgatatttggggccaagggacaatggtcaccgtctcttca

SEQ ID NO: 2 - protein, 126 aa, Artificial Sequence
  synthetic
QLQLQESGPGLVKPSETLSLTCTVSGASISSSRFYGGWIRQPPGKGLEWIGDIYYSGNTYYNPSLQSRVTISVDTSKNQFSLKLSSVTAADTAVYYCARHLMITFGGLIVEGFDIWGQGTMVTVSS

SEQ ID NO: 3 - DNA, 30 bp, Artificial Sequence
  synthetic
ggtgcctctatcagcagtagtcgtttctac

SEQ ID NO: 4 - protein, 10 aa, Artificial Sequence
  synthetic
GASISSSRFY

SEQ ID NO: 5 - DNA, 21 bp, Artificial Sequence
  synthetic
atctattatagtgggaatacc

SEQ ID NO: 6 - protein, 7 aa, Artificial Sequence
  synthetic
IYYSGNT

SEQ ID NO: 7 - DNA, 54 bp, Artificial Sequence
  synthetic
gcgagacaccttatgattacgtttgggggacttatcgtcgagggttttgatatt

SEQ ID NO: 8 - protein, 18 aa, Artificial Sequence
  synthetic
ARHLMITFGGLIVEGFDI

SEQ ID NO: 9 - DNA, 324 bp, Artificial Sequence
  synthetic
gacatccagatgacccagtctccatcctccctgtctgcatctgtaggagacagagtcaccatcacttgccgggcaagtcagagcattagcagctatttaaattggtatcagcagaaaccagggaaagcccctaagctcctgatctatgctgcatccagtttgcaaagtggggtcccgtcaaggttcagtggcagtggatctgggacagatttcactctcaccatcagcagtctgcaacctgaagattttgcaacttactactgtcaacagagttacagtacccctccgatcaccttcggccaagggacacgactggagattaaa

SEQ ID NO: 10 - protein, 108 aa, Artificial Sequence
  synthetic
DIQMTQSPSSLSASVGDRVTITCRASQSISSYLNWYQQKPGKAPKLLIYAASSLQSGVPSRFSGSGSGTDFTLTISSLQPEDFATYYCQQSYSTPPITFGQGTRLEIK

SEQ ID NO: 11 - DNA, 18 bp, Artificial Sequence
  synthetic
cagagcattagcagctat

SEQ ID NO: 12 - protein, 6 aa, Artificial Sequence
  synthetic
QSISSY

SEQ ID NO: 13 - DNA, 9 bp, Artificial Sequence
  synthetic
gctgcatcc

SEQ ID NO: 14 - protein, 3 aa, Artificial Sequence
  synthetic
AAS

SEQ ID NO: 15 - DNA, 30 bp, Artificial Sequence
  synthetic
caacagagttacagtacccctccgatcacc

SEQ ID NO: 16 - protein, 10 aa, Artificial Sequence
  synthetic
QQSYSTPPIT

SEQ ID NO: 17 - DNA, 366 bp, Artificial Sequence
  synthetic
caggtgcagctggtggagtctgggggaggcgtggtccagcctgggaggtccctgagactctcctgtgcagcctctggattcactttcagtagctatggcatccactgggtccgccaggctccaggcaaggggctggagtgggtggcagttatatcatatgatggaaataataaatactatgcagactccgtgaagggccgattcaccatctccagagacaattccaagaacacgctgtatctgcaaatgaacagcctgagagctgaggacacggctgtatattactgtgcgaaagatctatttttggagtggttatttcacggtatgggcgtctggggccaagggaccacggtcaccgtctcctca

SEQ ID NO: 18 - protein, 122 aa, Artificial Sequence
  synthetic
QVQLVESGGGVVQPGRSLRLSCAASGFTFSSYGIHWVRQAPGKGLEWVAVISYDGNNKYYADSVKGRFTISRDNSKNTLYLQMNSLRAEDTAVYYCAKDLFLEWLFHGMGVWGQGTTVTVSS

SEQ ID NO: 19 - DNA, 24 bp, Artificial Sequence
  synthetic
ggattcactttcagtagctatggc

SEQ ID NO: 20 - protein, 8 aa, Artificial Sequence
  synthetic
GFTFSSYG

SEQ ID NO: 21 - DNA, 24 bp, Artificial Sequence
  synthetic
atatcatatgatggaaataataaa

SEQ ID NO: 22 - protein, 8 aa, Artificial Sequence
  synthetic
ISYDGNNK

SEQ ID NO: 23 - DNA, 45 bp, Artificial Sequence
  synthetic
gcgaaagatctatttttggagtggttatttcacggtatgggcgtc

SEQ ID NO: 24 - protein, 15 aa, Artificial Sequence
  synthetic
AKDLFLEWLFHGMGV

SEQ ID NO: 25 - DNA, 372 bp, Artificial Sequence
  synthetic
cagctgcagctgcaggagtcgggcccaggactagtgaagccttcggagaccctgtccctcacctgcattgtctctggtggcgacatcaccagtagtagttattactggaactggatccgccagcccccagggaaagggctggagtggattgggaatatctattatagtggaagcaccaactacaacccgtccctcaagagtcgagtcaccatatccatagacacgtccaagagccagttctccctgaagctgaggtctgtgaccgccgcagacacggctgtttattactgtgcgagattattacgatattttgactggtcaaaaggataccttgactactggggccagggaaccctggtcaccgtctcctca

SEQ ID NO: 26 - protein, 124 aa, Artificial Sequence
  synthetic
QLQLQESGPGLVKPSETLSLTCIVSGGDITSSSYYWNWIRQPPGKGLEWIGNIYYSGSTNYNPSLKSRVTISIDTSKSQFSLKLRSVTAADTAVYYCARLLRYFDWSKGYLDYWGQGTLVTVSS

SEQ ID NO: 27 - DNA, 30 bp, Artificial Sequence
  synthetic
ggtggcgacatcaccagtagtagttattac

SEQ ID NO: 28 - protein, 10 aa, Artificial Sequence
  synthetic
GGDITSSSYY

SEQ ID NO: 29 - DNA, 21 bp, Artificial Sequence
  synthetic
atctattatagtggaagcacc

SEQ ID NO: 30 - protein, 7 aa, Artificial Sequence
  synthetic
IYYSGST

SEQ ID NO: 31 - DNA, 48 bp, Artificial Sequence
  synthetic
gcgagattattacgatattttgactggtcaaaaggataccttgactac

SEQ ID NO: 32 - protein, 16 aa, Artificial Sequence
  synthetic
ARLLRYFDWSKGYLDY

SEQ ID NO: 33 - DNA, 369 bp, Artificial Sequence
  synthetic
caggtgcagctggtggagtctgggggaggcatggtcaagcctggagggtccctgagactctcctgtgcagcctctggattcaccttcagtgactactatatgagctggatccgccaggctccagggaagggtctggagtggatttcacacattagtattactggtagcaccatatactacgcagactctgtgaagggccgattcaccatctccagggacaacgccaagaattcactgtatttggaaatgaacagactgagagacgaggacacggccgtatattactgtacgagagatgagccggatattgtactagtaaggtacggtatggacgtctggggccaagggaccacggtcaccgtctcctca

SEQ ID NO: 34 - protein, 123 aa, Artificial Sequence
  synthetic
QVQLVESGGGMVKPGGSLRLSCAASGFTFSDYYMSWIRQAPGKGLEWISHISITGSTIYYADSVKGRFTISRDNAKNSLYLEMNRLRDEDTAVYYCTRDEPDIVLVRYGMDVWGQGTTVTVSS

SEQ ID NO: 35 - DNA, 24 bp, Artificial Sequence
  synthetic
ggattcaccttcagtgactactat

SEQ ID NO: 36 - protein, 8 aa, Artificial Sequence
  synthetic
GFTFSDYY

SEQ ID NO: 37 - DNA, 24 bp, Artificial Sequence
  synthetic
attagtattactggtagcaccata

SEQ ID NO: 38 - protein, 8 aa, Artificial Sequence
  synthetic
ISITGSTI

SEQ ID NO: 39 - DNA, 48 bp, Artificial Sequence
  synthetic
acgagagatgagccggatattgtactagtaaggtacggtatggacgtc

SEQ ID NO: 40 - protein, 16 aa, Artificial Sequence
  synthetic
TRDEPDIVLVRYGMDV

SEQ ID NO: 41 - DNA, 351 bp, Artificial Sequence
  synthetic
gaggtgcagctggtggagtctgggggaagtgtggtacggcctggggaatccctgagactctcctgtgcagcctctggattcacatttgatgattatggcatgagctgggtccgccaagctccagggaaggggctggagtgggtctctggtattagttggaatggtggcatcacagtttatgcagactctgtgaagggccgattcaccgtctccagagacaacgccaagaactccctgtatctgcaaatgaacagtctgagagccgaggacacggccctctatcactgtgcgagagcccgttatggtggcgccgactactggggccagggaaccctggtcaccgtctcctca

SEQ ID NO: 42 - protein, 117 aa, Artificial Sequence
  synthetic
EVQLVESGGSVVRPGESLRLSCAASGFTFDDYGMSWVRQAPGKGLEWVSGISWNGGITVYADSVKGRFTVSRDNAKNSLYLQMNSLRAEDTALYHCARARYGGADYWGQGTLVTVSS

SEQ ID NO: 43 - DNA, 24 bp, Artificial Sequence
  synthetic
ggattcacatttgatgattatggc

SEQ ID NO: 44 - protein, 8 aa, Artificial Sequence
  synthetic
GFTFDDYG

SEQ ID NO: 45 - DNA, 24 bp, Artificial Sequence
  synthetic
attagttggaatggtggcatcaca

SEQ ID NO: 46 - protein, 8 aa, Artificial Sequence
  synthetic
ISWNGGIT

SEQ ID NO: 47 - DNA, 30 bp, Artificial Sequence
  synthetic
gcgagagcccgttatggtggcgccgactac

SEQ ID NO: 48 - protein, 10 aa, Artificial Sequence
  synthetic
ARARYGGADY

SEQ ID NO: 49 - DNA, 366 bp, Artificial Sequence
  synthetic
gaggtgcagctggtggagtctgggggagacttggtacagcctgggcggtccctgagactctcctgtgcagcctctggattcacctttagcagttttgccatgagctgggtccgccaggctccagggaggggactggagtgggtctcaagtctcagtgatagtggtgataacacatactacgcagactccgtgaagggccggttcaccatctccagagacaattccaaaaatacgttgtatctgcaaatgaacaacctgagagccgaggacacggccgtttattactgtgcgaaagatctcttttcggggtggttattccatggttttgatgtctggggccaagggacaatggtcaccgtctcttca

SEQ ID NO: 50 - protein, 122 aa, Artificial Sequence
  synthetic
EVQLVESGGDLVQPGRSLRLSCAASGFTFSSFAMSWVRQAPGRGLEWVSSLSDSGDNTYYADSVKGRFTISRDNSKNTLYLQMNNLRAEDTAVYYCAKDLFSGWLFHGFDVWGQGTMVTVSS

SEQ ID NO: 51 - DNA, 24 bp, Artificial Sequence
  synthetic
ggattcacctttagcagttttgcc

SEQ ID NO: 52 - protein, 8 aa, Artificial Sequence
  synthetic
GFTFSSFA

SEQ ID NO: 53 - DNA, 24 bp, Artificial Sequence
  synthetic
ctcagtgatagtggtgataacaca

SEQ ID NO: 54 - protein, 8 aa, Artificial Sequence
  synthetic
LSDSGDNT

SEQ ID NO: 55 - DNA, 45 bp, Artificial Sequence
  synthetic
gcgaaagatctcttttcggggtggttattccatggttttgatgtc

SEQ ID NO: 56 - protein, 15 aa, Artificial Sequence
  synthetic
AKDLFSGWLFHGFDV

SEQ ID NO: 57 - DNA, 351 bp, Artificial Sequence
  synthetic
caggttcagctggtgcagtctggacctgaagtgaaaaaacctggggcctcagtgaaggtctcttgtaagggttctggttacaccttttcctggtatggaatcagctggatccgacaggcccctggacacggccttgaatggatgggatggatcagcgcttccagtggtaatacaagatttgcacagaaggtccagggcagactcaccatgaccacagacacatcgacgagtacagcctacatggagctgaggagcctgagatctgacgacacggccgtttattactgtgcgagaacggggactcggccctttgactattggggccagggaaccctggtcaccgtctcctca

SEQ ID NO: 58 - protein, 117 aa, Artificial Sequence
  synthetic
QVQLVQSGPEVKKPGASVKVSCKGSGYTFSWYGISWIRQAPGHGLEWMGWISASSGNTRFAQKVQGRLTMTTDTSTSTAYMELRSLRSDDTAVYYCARTGTRPFDYWGQGTLVTVSS

SEQ ID NO: 59 - DNA, 24 bp, Artificial Sequence
  synthetic
ggttacaccttttcctggtatgga

SEQ ID NO: 60 - protein, 8 aa, Artificial Sequence
  synthetic
GYTFSWYG

SEQ ID NO: 61 - DNA, 24 bp, Artificial Sequence
  synthetic
atcagcgcttccagtggtaataca

SEQ ID NO: 62 - protein, 8 aa, Artificial Sequence
  synthetic
ISASSGNT

SEQ ID NO: 63 - DNA, 30 bp, Artificial Sequence
  synthetic
gcgagaacggggactcggccctttgactat

SEQ ID NO: 64 - protein, 10 aa, Artificial Sequence
  synthetic
ARTGTRPFDY

SEQ ID NO: 65 - DNA, 366 bp, Artificial Sequence
  synthetic
gaggtgcagctggtggagtctgggggaggcttggtccagccgggggggtccctgagactctcctgtacagcctctggattcaccttcagtagctatggtctgcactgggtccgccaggctccagggaagggactggaatatgtttcaagtattaatcataatgggggtagtaaatattatgcagactctgtgaagggcagattcaccatctccagagacaattcgaagaacacgctgtttcttcaaatgggcagcctgaaaactgaggacatggctgtttattactgtgcgagagatctctttttggagtggttattccatggttttgatatctggggccaagggacaatggtcaccgtctcttca

SEQ ID NO: 66 - protein, 122 aa, Artificial Sequence
  synthetic
EVQLVESGGGLVQPGGSLRLSCTASGFTFSSYGLHWVRQAPGKGLEYVSSINHNGGSKYYADSVKGRFTISRDNSKNTLFLQMGSLKTEDMAVYYCARDLFLEWLFHGFDIWGQGTMVTVSS

SEQ ID NO: 67 - DNA, 24 bp, Artificial Sequence
  synthetic
ggattcaccttcagtagctatggt

SEQ ID NO: 68 - protein, 8 aa, Artificial Sequence
  synthetic
GFTFSSYG

SEQ ID NO: 69 - DNA, 24 bp, Artificial Sequence
  synthetic
attaatcataatgggggtagtaaa

SEQ ID NO: 70 - protein, 8 aa, Artificial Sequence
  synthetic
INHNGGSK

SEQ ID NO: 71 - DNA, 45 bp, Artificial Sequence
  synthetic
gcgagagatctctttttggagtggttattccatggttttgatatc

SEQ ID NO: 72 - protein, 15 aa, Artificial Sequence
  synthetic
ARDLFLEWLFHGFDI

SEQ ID NO: 73 - DNA, 357 bp, Artificial Sequence
  synthetic
caggtgcagctgcaggagtcgggcccaggactggtgaagccttcacagaccctgtccctcacctgttctgtctctggtggctccataaacactggttcttacttctggacttggatccgccagcacccaggggagggcctggagtggattgggtacatctattacaatggagacacctactacaatccgtccctcaagagtcgagttaccttatcactagacacgtctaagaaccagttctccctgaagctgaactctctgactgccggggacacggccgtttattactgtgcgagaagtgactggaactccctttttgaccactggggccaggggaccctggtcaccgtctcctca

SEQ ID NO: 74 - protein, 119 aa, Artificial Sequence
  synthetic
QVQLQESGPGLVKPSQTLSLTCSVSGGSINTGSYFWTWIRQHPGEGLEWIGYIYYNGDTYYNPSLKSRVTLSLDTSKNQFSLKLNSLTAGDTAVYYCARSDWNSLFDHWGQGTLVTVSS

SEQ ID NO: 75 - DNA, 30 bp, Artificial Sequence
  synthetic
ggtggctccataaacactggttcttacttc

SEQ ID NO: 76 - protein, 10 aa, Artificial Sequence
  synthetic
GGSINTGSYF

SEQ ID NO: 77 - DNA, 21 bp, Artificial Sequence
  synthetic
atctattacaatggagacacc

SEQ ID NO: 78 - protein, 7 aa, Artificial Sequence
  synthetic
IYYNGDT

SEQ ID NO: 79 - DNA, 33 bp, Artificial Sequence
  synthetic
gcgagaagtgactggaactccctttttgaccac

SEQ ID NO: 80 - protein, 11 aa, Artificial Sequence
  synthetic
ARSDWNSLFDH

SEQ ID NO: 81 - DNA, 324 bp, Artificial Sequence
  synthetic
gaaattgtgttgacgcagtctccaggcaccctgtctttgtctccaggggaaagagccaccctctcctgcagggccagtcagagtgttagcagcagctacttagcctggtaccagcagaaacctggccaggctcccaggctcctcatctatggtgcatccagcagggccactggcatcccagacaggttcagtggcagtgggtctgggacagacttcactctcaccatcagcagactggagcctgaagattttgcagtgtattactgtcagcagtatggtagctcaccttggacgttcggccaagggaccaaggtggaaatcaaa

SEQ ID NO: 82 - protein, 108 aa, Artificial Sequence
  synthetic
EIVLTQSPGTLSLSPGERATLSCRASQSVSSSYLAWYQQKPGQAPRLLIYGASSRATGIPDRFSGSGSGTDFTLTISRLEPEDFAVYYCQQYGSSPWTFGQGTKVEIK

SEQ ID NO: 83 - DNA, 21 bp, Artificial Sequence
  synthetic
cagagtgttagcagcagctac

SEQ ID NO: 84 - protein, 7 aa, Artificial Sequence
  synthetic
QSVSSSY

SEQ ID NO: 85 - DNA, 9 bp, Artificial Sequence
  synthetic
ggtgcatcc

SEQ ID NO: 86 - protein, 3 aa, Artificial Sequence
  synthetic
GAS

SEQ ID NO: 87 - DNA, 27 bp, Artificial Sequence
  synthetic
cagcagtatggtagctcaccttggacg

SEQ ID NO: 88 - protein, 9 aa, Artificial Sequence
  synthetic
QQYGSSPWT

SEQ ID NO: 89 - protein, 1165 aa, Artificial Sequence
  hLEPR P48357
MICQKFCVVLLHWEFIYVITAFNLSYPITPWRFKLSCMPPNSTYDYFLLPAGLSKNTSNSNGHYETAVEPKFNSSGTHFSNLSKTTFHCCFRSEQDRNCSLCADNIEGKTFVSTVNSLVFQQIDANWNIQCWLKGDLKLFICYVESLFKNLFRNYNYKVHLLYVLPEVLEDSPLVPQKGSFQMVHCNCSVHECCECLVPVPTAKLNDTLLMCLKITSGGVIFQSPLMSVQPINMVKPDPPLGLHMEITDDGNLKISWSSPPLVPFPLQYQVKYSENSTTVIREADKIVSATSLLVDSILPGSSYEVQVRGKRLDGPGIWSDWSTPRVFTTQDVIYFPPKILTSVGSNVSFHCIYKKENKIVPSKEIVWWMNLAEKIPQSQYDVVSDHVSKVTFFNLNETKPRGKFTYDAVYCCNEHECHHRYAELYVIDVNINISCETDGYLTKMTCRWSTSTIQSLAESTLQLRYHRSSLYCSDIPSIHPISEPKDCYLQSDGFYECIFQPIFLLSGYTMWIRINHSLGSLDSPPTCVLPDSVVKPLPPSSVKAEITINIGLLKISWEKPVFPENNLQFQIRYGLSGKEVQWKMYEVYDAKSKSVSLPVPDLCAVYAVQVRCKRLDGLGYWSNWSNPAYTVVMDIKVPMRGPEFWRIINGDTMKKEKNVTLLWKPLMKNDSLCSVQRYVINHHTSCNGTWSEDVGNHTKFTFLWTEQAHTVTVLAINSIGASVANFNLTFSWPMSKVNIVQSLSAYPLNSSCVIVSWILSPSDYKLMYFIIEWKNLNEDGEIKWLRISSSVKKYYIHDHFIPIEKYQFSLYPIFMEGVGKPKIINSFTQDDIEKHQSDAGLYVIVPVIISSSILLLGTLLISHQRMKKLFWEDVPNPKNCSWAQGLNFQKPETFEHLFIKHTASVTCGPLLLEPETISEDISVDTSWKNKDEMMPTTVVSLLSTTDLEKGSVCISDQFNSVNFSEAEGTEVTYEDESQRQPFVKYATLISNSKPSETGEEQGLINSSVTKCFSSKNSPLKDSFSNSSWEIEAQAFFILSDQHPNIISPHLTFSEGLDELLKLEGNFPEENNDKKSIYYLGVTSIKKRESGVLLTDKSRVSCPFPAPCLFTDIRVLQDSCSHFVENNINLGTSSKKTFASYMPQFQTCSTQTHKIMENKMCDLTV

SEQ ID NO: 90 - protein, 846 aa, Artificial Sequence
  hLEPR-mmh aa 1-818: F22-D839 of P48357 aa 819-846: myc-myc-hexahistidine tag
FNLSYPITPWRFKLSCMPPNSTYDYFLLPAGLSKNTSNSNGHYETAVEPKFNSSGTHFSNLSKTTFHCCFRSEQDRNCSLCADNIEGKTFVSTVNSLVFQQIDANWNIQCWLKGDLKLFICYVESLFKNLFRNYNYKVHLLYVLPEVLEDSPLVPQKGSFQMVHCNCSVHECCECLVPVPTAKLNDTLLMCLKITSGGVIFQSPLMSVQPINMVKPDPPLGLHMEITDDGNLKISWSSPPLVPFPLQYQVKYSENSTTVIREADKIVSATSLLVDSILPGSSYEVQVRGKRLDGPGIWSDWSTPRVFTTQDVIYFPPKILTSVGSNVSFHCIYKKENKIVPSKEIVWWMNLAEKIPQSQYDVVSDHVSKVTFFNLNETKPRGKFTYDAVYCCNEHECHHRYAELYVIDVNINISCETDGYLTKMTCRWSTSTIQSLAESTLQLRYHRSSLYCSDIPSIHPISEPKDCYLQSDGFYECIFQPIFLLSGYTMWIRINHSLGSLDSPPTCVLPDSVVKPLPPSSVKAEITINIGLLKISWEKPVFPENNLQFQIRYGLSGKEVQWKMYEVYDAKSKSVSLPVPDLCAVYAVQVRCKRLDGLGYWSNWSNPAYTVVMDIKVPMRGPEFWRIINGDTMKKEKNVTLLWKPLMKNDSLCSVQRYVINHHTSCNGTWSEDVGNHTKFTFLWTEQAHTVTVLAINSIGASVANFNLTFSWPMSKVNIVQSLSAYPLNSSCVIVSWILSPSDYKLMYFIIEWKNLNEDGEIKWLRISSSVKKYYIHDHFIPIEKYQFSLYPIFMEGVGKPKIINSFTQDDIEKHQSDEQKLISEEDLGGEQKLISEEDLHHHHHH

SEQ ID NO: 91 - protein, 1051 aa, Artificial Sequence
  hLEPR-mFc aa 1-818: F22-D839 of P48357 aa 819-1051: mouse IgG2a (E98-K330 of P01863)
FNLSYPITPWRFKLSCMPPNSTYDYFLLPAGLSKNTSNSNGHYETAVEPKFNSSGTHFSNLSKTTFHCCFRSEQDRNCSLCADNIEGKTFVSTVNSLVFQQIDANWNIQCWLKGDLKLFICYVESLFKNLFRNYNYKVHLLYVLPEVLEDSPLVPQKGSFQMVHCNCSVHECCECLVPVPTAKLNDTLLMCLKITSGGVIFQSPLMSVQPINMVKPDPPLGLHMEITDDGNLKISWSSPPLVPFPLQYQVKYSENSTTVIREADKIVSATSLLVDSILPGSSYEVQVRGKRLDGPGIWSDWSTPRVFTTQDVIYFPPKILTSVGSNVSFHCIYKKENKIVPSKEIVWWMNLAEKIPQSQYDVVSDHVSKVTFFNLNETKPRGKFTYDAVYCCNEHECHHRYAELYVIDVNINISCETDGYLTKMTCRWSTSTIQSLAESTLQLRYHRSSLYCSDIPSIHPISEPKDCYLQSDGFYECIFQPIFLLSGYTMWIRINHSLGSLDSPPTCVLPDSVVKPLPPSSVKAEITINIGLLKISWEKPVFPENNLQFQIRYGLSGKEVQWKMYEVYDAKSKSVSLPVPDLCAVYAVQVRCKRLDGLGYWSNWSNPAYTVVMDIKVPMRGPEFWRIINGDTMKKEKNVTLLWKPLMKNDSLCSVQRYVINHHTSCNGTWSEDVGNHTKFTFLWTEQAHTVTVLAINSIGASVANFNLTFSWPMSKVNIVQSLSAYPLNSSCVIVSWILSPSDYKLMYFIIEWKNLNEDGEIKWLRISSSVKKYYIHDHFIPIEKYQFSLYPIFMEGVGKPKIINSFTQDDIEKHQSDEPRGPTIKPCPPCKCPAPNLLGGPSVFIFPPKIKDVLMISLSPIVTCVVVDVSEDDPDVQISWFVNNVEVHTAQTQTHREDYNSTLRVVSALPIQHQDWMSGKEFKCKVNNKDLPAPIERTISKPKGSVRAPQVYVLPPPEEEMTKKQVTLTCMVTDFMPEDIYVEWTNNGKTELNYKNTEPVLDSDGSYFMYSKLRVEKKNWVERNSYSCSVVHEGLHNHHTTKSFSRTPGK

SEQ ID NO: 92 - protein, 1045 aa, Artificial Sequence
  hLEPR-hFc aa 1-818: F22-D839 of P48357 aa 819-1045: human IgG1 (D104-K330 of P01857)
FNLSYPITPWRFKLSCMPPNSTYDYFLLPAGLSKNTSNSNGHYETAVEPKFNSSGTHFSNLSKTTFHCCFRSEQDRNCSLCADNIEGKTFVSTVNSLVFQQIDANWNIQCWLKGDLKLFICYVESLFKNLFRNYNYKVHLLYVLPEVLEDSPLVPQKGSFQMVHCNCSVHECCECLVPVPTAKLNDTLLMCLKITSGGVIFQSPLMSVQPINMVKPDPPLGLHMEITDDGNLKISWSSPPLVPFPLQYQVKYSENSTTVIREADKIVSATSLLVDSILPGSSYEVQVRGKRLDGPGIWSDWSTPRVFTTQDVIYFPPKILTSVGSNVSFHCIYKKENKIVPSKEIVWWMNLAEKIPQSQYDVVSDHVSKVTFFNLNETKPRGKFTYDAVYCCNEHECHHRYAELYVIDVNINISCETDGYLTKMTCRWSTSTIQSLAESTLQLRYHRSSLYCSDIPSIHPISEPKDCYLQSDGFYECIFQPIFLLSGYTMWIRINHSLGSLDSPPTCVLPDSVVKPLPPSSVKAEITINIGLLKISWEKPVFPENNLQFQIRYGLSGKEVQWKMYEVYDAKSKSVSLPVPDLCAVYAVQVRCKRLDGLGYWSNWSNPAYTVVMDIKVPMRGPEFWRIINGDTMKKEKNVTLLWKPLMKNDSLCSVQRYVINHHTSCNGTWSEDVGNHTKFTFLWTEQAHTVTVLAINSIGASVANFNLTFSWPMSKVNIVQSLSAYPLNSSCVIVSWILSPSDYKLMYFIIEWKNLNEDGEIKWLRISSSVKKYYIHDHFIPIEKYQFSLYPIFMEGVGKPKIINSFTQDDIEKHQSDDKTHTCPPCPAPELLGGPSVFLFPPKPKDTLMISRTPEVTCVVVDVSHEDPEVKFNWYVDGVEVHNAKTKPREEQYNSTYRVVSVLTVLHQDWLNGKEYKCKVSNKALPAPIEKTISKAKGQPREPQVYTLPPSRDELTKNQVSLTCLVKGFYPSDIAVEWESNGQPENNYKTTPPVLDSDGSFFLYSKLTVDKSRWQQGNVFSCSVMHEALHNHYTQKSLSLSPGK

SEQ ID NO: 93 - protein, 844 aa, Artificial Sequence
  MfLEPR-mmh aa 1-816: Macaca fascicularis LEPR (F22-D837 of XP_005543194.1 with a T827A substitution) aa 817-844: myc-myc-hexahistidine tag
FNLSYPITPWRFKLSCMPPNSTYDYFLLPAGLSKNTSNLNGHYETAVEFNSSDTHFSNLSKTTFHCCFRSEQDRNCSLCADNIEGKTFVSTVNSSVFQQMGANWNIQCWLKGDLKLFICYVESLFKNPFKNYKHKVHLLYVLPEVLEDSPLVPQKGSFQMVHCNCSVHERCECLVPVPTAKLNDTLLMCLKITSGGVIFQSPLMSVQPINMVKPDPPLGLRMEITDDGNLKISWSSPPLVPFPLQYEVKYSENSTTVIREADKIVSATSLLVDGILPGSSYEVQVRGKRLDGPGIWSDWSTPHVFTTQDVIYFPPKILTSVGSNVSFHCIYKNENKIVSSKKIVWWMNLAEKIPQSQYDVVSDHVSKVTFFNLNETKPRGKFTYDAVYCCNEHECHHRYAELYVIDVNINISCETDGHLTKMTCRWSTNTIQSLAGSTLQLRYRRSSLYCFDIPSIHPISKPKDCYLQSDGFYECVFQPIFLLSGYTMWIRINHPLGSLDSPPTCVLPDSVVKPLPPSSVKAEIIKNIGLLKISWEKPVFPENNLQFQIRYGLSGKEIQWKMYDVYDAKSKSVSLPVPDFCAVYAVQVRCKRSDGLGLWSNWSNPAYTVVMDIKVPMRGPEFWRIINGDTMKKEKNVTLLWKPLMKNDSLCSVQRYVINHHTSCNGTWSEDVGNHTKFTFLWTEQAHTVTVLAINSIGASVANFNLTFSWPMSKVNIVQSLSAYPLNSSCVILSWILSPSDYKLMYFIIEWKNLNEDGEIKWLRISSSVKKYYIHDHFIPIEKYQFSLYPIFMEGVGKPKIINSFAQDNTEKHQNDEQKLISEEDLGGEQKLISEEDLHHHHHH

SEQ ID NO: 94 - protein, 846 aa, Artificial Sequence
  mLEPR-mmh aa 1-818: mouse LEPR (L22-G839 of NP_666258.2) aa 819-846: myc-myc-hexahistidine tag
LNLAYPISPWKFKLFCGPPNTTDDSFLSPAGAPNNASALKGASEAIVEAKFNSSGIYVPELSKTVFHCCFGNEQGQNCSALTDNTEGKTLASVVKASVFRQLGVNWDIECWMKGDLTLFICHMEPLPKNPFKNYDSKVHLLYDLPEVIDDSPLPPLKDSFQTVQCNCSLRGCECHVPVPRAKLNYALLMYLEITSAGVSFQSPLMSLQPMLVVKPDPPLGLHMEVTDDGNLKISWDSQTMAPFPLQYQVKYLENSTIVREAAEIVSATSLLVDSVLPGSSYEVQVRSKRLDGSGVWSDWSSPQVFTTQDVVYFPPKILTSVGSNASFHCIYKNENQIISSKQIVWWRNLAEKIPEIQYSIVSDRVSKVTFSNLKATRPRGKFTYDAVYCCNEQACHHRYAELYVIDVNINISCETDGYLTKMTCRWSPSTIQSLVGSTVQLRYHRRSLYCPDSPSIHPTSEPKNCVLQRDGFYECVFQPIFLLSGYTMWIRINHSLGSLDSPPTCVLPDSVVKPLPPSNVKAEITVNTGLLKVSWEKPVFPENNLQFQIRYGLSGKEIQWKTHEVFDAKSKSASLLVSDLCAVYVVQVRCRRLDGLGYWSNWSSPAYTLVMDVKVPMRGPEFWRKMDGDVTKKERNVTLLWKPLTKNDSLCSVRRYVVKHRTAHNGTWSEDVGNRTNLTFLWTEPAHTVTVLAVNSLGASLVNFNLTFSWPMSKVSAVESLSAYPLSSSCVILSWTLSPDDYSLLYLVIEWKILNEDDGMKWLRIPSNVKKFYIHDNFIPIEKYQFSLYPVFMEGVGKPKIINGFTKDAIDKQQNDAGEQKLISEEDLGGEQKLISEEDLHHHHHH

SEQ ID NO: 95 - protein, 846 aa, Artificial Sequence
  rLEPR-mmh aa 1-818: rat LEPR (L22-G839 of NP_036728.1) aa 819-846: myc-myc-hexahistidine tag
LNLAYPTSPWRFKLFCAPPSTTDDSFLSPAGVPNNTSSLKGASEALVEAKFNSTGIYVSELSKTIFHCCFGNEQGQNCSALTGNTEGKTLASVVKPLVFRQLGVNWDIECWMKGDLTLFICHMEPLLKNPFKNYDSKVHLLYDLPEVIDDLPLPPLKDSFQTVQCNCSVRECECHVPVPRAKVNYALLMYLEITSAGVSFQSPLMSLQPMLVVKPDPPLGLRMEVTDDGNLKISWDSQTKAPFPLQYQVKYLENSTIVREAAEIVSDTSLLVDSVLPGSSYEVQVRSKRLDGSGVWSDWSLPQLFTTQDVMYFPPKILTSVGSNASFCCIYKNENQTISSKQIVWWMNLAEKIPETQYNTVSDHISKVTFSNLKATRPRGKFTYDAVYCCNEQACHHRYAELYVIDVNINISCETDGYLTKMTCRWSPSTIQSLVGSTVQLRYHRRSLYCPDNPSIRPTSELKNCVLQTDGFYECVFQPIFLLSGYTMWIRINHSLGSLDSPPTCVLPDSVVKPLPPSNVKAEITINTGLLKVSWEKPVFPENNLQFQIRYGLNGKEIQWKTHEVFDAKSKSASLPVSDLCAVYVVQVRCRRLDGLGYWSNWSSPAYTLVMDVKVPMRGPEFWRIMDGDITKKERNVTLLWKPLMKNDSLCSVRRYVVKHRTAHNGTWSQDVGNQTNLTFLWAESAHTVTVLAINSIGASLVNFNLTFSWPMSKVNAVQSLSAYPLSSSCVILSWTLSPNDYSLLYLVIEWKNLNDDDGMKWLRIPSNVNKYYIHDNFIPIEKYQFSLYPVFMEGVGKPKIINGFTKDDIAKQQNDAGEQKLISEEDLGGEQKLISEEDLHHHHHH